European Patent Application EP 4 813 401 A1, published September 30, 2026. Title: 重组溶瘤病毒和大分子抗体抗癌药联合治疗肿瘤的方法. Applicant: JOINT BIOSCIENCES (SH) LTD. The sequence listing filed with the application follows.

SEQUENCE LISTING (60 sequences)

SEQ ID NO: 1 - protein, 229 aa, unidentified
  source 1..229: note = Indiana MuddSummer subtype of VSV virus
MSSLKKILGLKGKGKKSKKLGIAPPPYEEDTNMEYAPSAPIDKSYFGVNEMDTHDPNQLRYEKFFFTVKMTVRSNRPFRTYSDVAAAVSHWDHMYIGMAGKRPFYKILAFLGSSNLKATPAVLADQGQPEYHAHCEGRAYLPHRMGKTPPMLNVPEHFRRPFNIGLYKGTIELTMTIYDDESLEAAPMIWDHFNSSKFSDFREKALMFGLIVEKKASGAWVLDSVSHFK

SEQ ID NO: 2 - protein, 229 aa, synthetic construct
MSSLKKILGLKGKGKKSKKLGIAPPPYEEDTNMEYAPSAPIDKSYFGVNERDTHDPNQLRYEKFFFTVKMTVRSNRPFRTYSDVAAAVSHWDHMYIGMAGKRPFYKILAFLGSSNLKATPAVLADQGQPEYHAHCEGRAYLPHRMGKTPPMLNVPEHFRRPFNIGLYKGTIELTMTIYDDESLEAAPMIWDHFNSSKFSDFREKALMFGLIVEKKASGAWFLDSVRHFK

SEQ ID NO: 3 - protein, 229 aa, synthetic construct
MSSLKKILGLKGKGKKSKKLGIAPPPYEEDTSMEYAPSAPIDKSYFGVDERDTYDPNQLRYEKFFFTVKMTVRSNRPFRTYSDVAAAVSHWDHMYIGMAGKRPFYKILAFLGSSNLKATPAVLADQGQPEYHAHCEGRAYLPHRMGKTPPMLNVPEHFRRPFNIGLYKGTIELTMTIYDDESLEAAPMIWDHFNSSKFSDFREKALMFGLIVEKKASGAWFLDSIRHFK

SEQ ID NO: 4 - protein, 228 aa, synthetic construct
MSSLKKILGLKGKGKKSKKLGIAPPPYEEDTSMEYAPSAPIDKSYFGVDERDTYDPNQLRYEKFFFTVKMTVRSNRPFRTYSDVAAAVSHWDHMYIGMAGKRPFYKILAFGSSNLKATPAVLADQGQPEYHAHCEGRAYLPHRMGKTPPMLNVPEHFRRPFNIGLYKGTIELTMTIYDDESLEAAPMIWDHFNSSKFSDFREKALMFGLIVEKKASGAWFLDSIRHFK

SEQ ID NO: 5 - protein, 229 aa, synthetic construct
MSSLKKILGLKGKGKKSKKLGIAPPPYEEDTSMEYAPSAPIDKSYFGVDERDTYDPNQLRYEKFFFTVKMTVRSNRPFRTYSDVAAAVSHWDHMYIGMAGKRPFYKILAFAGSSNLKATPAVLADQGQPEYHAHCEGRAYLPHRMGKTPPMLNVPEHFRRPFNIGLYKGTIELTMTIYDDESLEAAPMIWDHFNSSKFSDFREKALMFGLIVEKKASGAWFLDSIRHFK

SEQ ID NO: 6 - protein, 229 aa, synthetic construct
MSSLKKILGLKGKGKKSKKLEIAPPPYEEDTSMEYAPSAPIDKSYFGVDERDTYDPNQLRYEKFFFTVKMTVRSNRPFRTYSDVAAAVSHWDHMYIGMAGKRPFYKILAFLGSSNLKATPAVLADQGQPEYHAHCEGRAYLPHRMGKTPPMLNVPEHFRRPFNIGLYKGTIELTMTIYDDESLEAAPMIWDHFNSSKFSDFREKALMFGLIVEKKASGAWFLDSIRHFK

SEQ ID NO: 7 - protein, 229 aa, synthetic construct
MSSLKKILGLKGKGKKSKKLEIAPPPYEEDTSAEYAPSAPIDKSYFGVDERDTYDPNQLRYEKFFFTVKMTVRSNRPFRTYSDVAAAVSHWDHMYIGMAGKRPFYKILAFLGSSNLKATPAVLADQGQPEYHAHCEGRAYLPHRMGKTPPMLNVPEHFRRPFNIGLYKGTIELTMTIYDDESLEAAPMIWDHFNSSKFSDFREKALMFGLIVEKKASGAWFLDSIRHFK

SEQ ID NO: 8 - protein, 229 aa, synthetic construct
MSSLKKILGLKGKGKKSKKLEIAPPPYEEDTSAEYAPSAPIDKSYFGVDERDTYDPNQLRYEKFFFTVKMTVRSNRPFRTYSDVAAAVSHWDHMYIGMAGKRPFYKILAFLGSSNLKATPAVLADQGQPEYHTHCEGRAYLPHRMGKTPPMLNVPEHFRRPFNIGLYKGTIELTMTIYDDESLEAAPMIWDHFNSSKFSDFREKALMFGLIVEKKASGAWFLDSIRHFK

SEQ ID NO: 9 - protein, 229 aa, synthetic construct
MSSLKKILGLKGKGKKSKKLGIAPPPYEEDTNAEYAPSAPIDKSYFGVNERDTHDPNQLRYEKFFFTVKMTVRSNRPFRTYSDVAAAVSHWDHMYIGMAGKRPFYKILAFLGSSNLKATPAVLADQGQPEYHAHCEGRAYLPHRMGKTPPMLNVPEHFRRPFNIGLYKGTIELTMTIYDDESLEAAPMIWDHFNSSKFSDFREKALMFGLIVEKKASGAWFLDSVRHFK

SEQ ID NO: 10 - protein, 229 aa, synthetic construct
MSSLKKILGLKGKGKKSKKLGIAPPPYEEDTNAEYAPSAPIDKSYFGVNERDTHDPNQLRYEKFFFTVKMTVRSNRPFRTYSDVAAAVSHWDHMYIGMAGKRPFYKILAFLGSSNLKATPAVLADQGQPEYHTHCEGRAYLPHRMGKTPPMLNVPEHFRRPFNIGLYKGTIELTMTIYDDESLEAAPMIWDHFNSSKFSDFREKALMFGLIVEKKASGAWFLDSVRHFK

SEQ ID NO: 11 - protein, 229 aa, synthetic construct
MSSLKKILGLKGKGKKSKKLGIAPPPYEEDTNMEYAPSAPIDKSYFGVNERDTHDPNQLRYEKFFFTVKMTVRSNRPFRTYSDVAAAVSHWDHMYIGMAGKRPFYKILAFLGSSNLKATPAVLADQGQPEYHTHCEGRAYLPHRMGKTPPMLNVPEHFRRPFNIGLYKGTIELTMTIYDDESLEAAPMIWDHFNSSKFSDFREKALMFGLIVEKKASGAWFLDSVRHFK

SEQ ID NO: 12 - protein, 511 aa, unidentified
  source 1..511: note = Indiana MuddSummer subtype of VSV virus
MKCLLYLAFLFIGVNCKFTIVFPHNQKGNWKNVPSNYHYCPSSSDLNWHNDLVGTALQVKMPKSHKAIQADGWMCHASKWVTTCDFRWYGPKYITHSIRSFTPSVEQCKESIEQTKQGTWLNPGFPPQSCGYATVTDAEAAIVQVTPHHVLVDEYTGEWVDSQFINGKCSNDICPTVHNSTTWHSDYKVKGLCDSNLISMDITFFSEDGELSSLGKKGTGFRSNYFAYETGDKACKMQYCKHWGVRLPSGVWFEMADKDLFAAARFPECPEGSSISAPSQTSVDVSLIQDVERILDYSLCQETWSKIRAGLPISPVDLSYLAPKNPGTGPVFTIINGTLKYFETRYIRVDIAAPILSRMVGMISGTTTERVLWDDWAPYEDVEIGPNGVLRTSSGYKFPLYMIGHGMLDSDLHLSSKAQVFEHPHIQDAASQLPDGETLFFGDTGLSKNPIEFVEGWFSSWKSSIASFFFTIGLIIGLFLVLRVGIYLCIKLKHTKKRQIYTDIEMNRLGK

SEQ ID NO: 13 - protein, 511 aa, synthetic construct
MKCLLYLAFLFIGVNCKFTIVFPHNQKGNWKNVPSNYHYCPSSSDLNWHNDLIGTALQVKMPKSHKAIQADGWMCHASKWVTTCDFRWYGPKYITHSIRSFTPSVEQCKESIEQTKQGTWLNPGFPPQSCGYATVTDAEAVIVQVTPHHVLVDEYTGEWVDSQFINGKCSNYICPTVHNSTTWHSDYKVKGLCDSNLISMDITFFSEDGELSSLGKEGTGFRSNYFAYETGGKACKMQYCKHWGVRLPSGVWFEMADKDLFAAARFPECPEGSSISAPSQTSVDVSLIQDVERILDYSLCQETWSKIRAGLPISPVDLSYLAPKNPGTGPAFTIINGTLKYFETRYIRVDIAAPILSRMVGMISGTTTERELWDDWAPYEDVEIGPNGVLRTSSGYKFPLYMIGHGMLDSDLHLSSKAQVFEHPHIQDAASQLPDDESLFFGDTGLSKNPIELVEGWFSSWKSSIASFFFIIGLIIGLFLVLRVGIHLCIKLKHTKKRQIYTDIEMNRLGK

SEQ ID NO: 14 - protein, 422 aa, unidentified
  source 1..422: note = Indiana MuddSummer subtype of VSV virus
MSVTVKRIIDNTVIVPKLPANEDPVEYPADYFRKSKEIPLYINTTKSLSDLRGYVYQGLKSGNVSIIHVNSYLYGALKDIRGKLDKDWSSFGINIGKAGDTIGIFDLVSLKALDGVLPDGVSDASRTSADDKWLPLYLLGLYRVGRTQMPEYRKRLMDGLTNQCKMINEQFEPLVPEGRDIFDVWGNDSNYTKIVAAVDMFFHMFKKHECASFRYGTIVSRFKDCAALATFGHLCKITGMSTEDVTTWILNREVADEMVQMMLPGQEIDKADSYMPYLIDFGLSSKSPYSSVKNPAFHFWGQLTALLLRSTRARNARQPDDIEYTSLTTAGLLYAYAVGSSADLAQQFCVGDSKYTPDDSTGGLTTNAPPQGRDVVEWLGWFEDQNRKPTPDMMQYAKRAVMSLQGLREKTIGKYAKSEFDK

SEQ ID NO: 15 - protein, 422 aa, synthetic construct
MSVTVKRIIDNTVVVPKLPANEDPVEYPADYFRKSKEIPLYINTTKSLSDLRGYVYQGLKSGNVSIIHVNSYLYGALKDIRGKLDKDWSSFGINIGKAGDTIGIFDLVSLKALDGVLPDGVSDASRTSADDKWLPLYLLGLYRVGRTQMPEYRKKLMDGLTNQCKMINEQFEPLVPEGRDIFDVWGNDSNYTKIVAAVDMFFHMFKKHECASFRYGTIVSRFKDCAALATFGHLCKITGMSTEDVTTWILNREVADEMVQMMLPGQEIDKADSYMPYLIDFGLSSKSPYSSVKNPAFHFWGQLTALLLRSTRARNARQPDDIEYTSLTTAGLLYAYAVGSSADLAQQFCVGDNKYTPDDSTGGLTTNAPPQGRDVVEWLGWFEDQNRKPTPDMMQYAKRAVMSLQGLREKTIGKYAKSEFDK

SEQ ID NO: 16 - protein, 265 aa, unidentified
  source 1..265: note = Indiana MuddSummer subtype of VSV virus
MDNLTKVREYLKSYSRLDQAVGEIDEIEAQRAEKSNYELFQEDGVEEHTRPSYFQAADDSDTESEPEIEDNQGLYVPDPEAEQVEGFIQGPLDDYADEDVDVVFTSDWKQPELESDEHGKTLRLTLPEGLSGEQKSQWLLTIKAVVQSAKHWNLAECTFEASGEGVIIKKRQITPDVYKVTPVMNTHPYQSEAVSDVWSLSKTSMTFQPKKASLQPLTISLDELFSSRGEFISVGGNGRMSHKEAILLGLRYKKLYNQARVKYSL

SEQ ID NO: 17 - protein, 265 aa, synthetic construct
MDNLTKVREYLKSYSRLDQAVGEIDEIEAQRAEKSNYELFQEDGVEEHTKPSYFQAADDSDTESEPEIEDNQGLYAPDPEAEQVEGFIQGPLDDYADEEVDVVFTSDWKQPELESDEHGKTLRLTSPEGLSGEQKSQWLSTIKAVVQSAKYWNLAECTFEASGEGVIMKERQITPDVYKVTPVMNTHPSQSEAVSDVWSLSKTSMTFQPKKASLQPLTISLDELFSSRGEFISVGGDGRMSHKEAILLGLRYKKLYNQARVKYSL

SEQ ID NO: 18 - protein, 2109 aa, unidentified
  source 1..2109: note = Indiana MuddSummer subtype of VSV virus
MEVHDFETDEFNDFNEDDYATREFLNPDERMTYLNHADYNLNSPLISDDIDNLIRKFNSLPIPSMWDSKNWDGVLEMLTSCQANPISTSQMHKWMGSWLMSDNHDASQGYSFLHEVDKEAEITFDVVETFIRGWGNKPIEYIKKERWTDSFKILAYLCQKFLDLHKLTLILNAVSEVELLNLARTFKGKVRRSSHGTNICRIRVPSLGPTFISEGWAYFKKLDILMDRNFLLMVKDVIIGRMQTVLSMVCRIDNLFSEQDIFSLLNIYRIGDKIVERQGNFSYDLIKMVEPICNLKLMKLARESRPLVPQFPHFENHIKTSVDEGAKIDRGIRFLHDQIMSVKTVDLTLVIYGSFRHWGHPFIDYYTGLEKLHSQVTMKKDIDVSYAKALASDLARIVLFQQFNDHKKWFVNGDLLPHDHPFKSHVKENTWPTAAQVQDFGDKWHELPLIKCFEIPDLLDPSIIYSDKSHSMNRSEVLKHVRMNPNIPIPSKKVLQTMLDTKATNWKEFLKEIDEKGLDDDDLIIGLKGKERELKLAGRFFSLMSWKLREYFVITEYLIKTHFVPMFKGLTMADDLTAVIKKMLDSSSGQGLKSYEAICIANHIDYEKWNNHQRKLSNGPVFRVMGQFLGYPSLIERTHEFFEKSLIYYNGRPDLMRVHNNTLINSTSQRVCWQGQEGGLEGLRQKGWSILNLLVIQREAKIRNTAVKVLAQGDNQVICTQYKTKKSRNVVELQGALNQMVSNNEKIMTAIKIGTGKLGLLINDDETMQSADYLNYGKIPIFRGVIRGLETKRWSRVTCVTNDQIPTCANIMSSVSTNALTVAHFAENPINAMIQYNYFGTFARLLLMMHDPALRQSLYEVQDKIPGLHSSTFKYAMLYLDPSIGGVSGMSLSRFLIRAFPDPVTESLSFWRFIHVHARSEHLKEMSAVFGNPEIAKFRITHIDKLVEDPTSLNIAMGMSPANLLKTEVKKCLIESRQTIRNQVIKDATIYLYHEEDRLRSFLWSINPLFPRFLSEFKSGTFLGVADGLISLFQNSRTIRNSFKKKYHRELDDLIVRSEVSSLTHLGKLHLRRGSCKMWTCSATHADTLRYKSWGRTVIGTTVPHPLEMLGPQHRKETPCAPCNTSGFNYVSVHCPDGIHDVFSSRGPLPAYLGSKTSESTSILQPWERESKVPLIKRATRLRDAISWFVEPDSKLAMTILSNIHSLTGEEWTKRQHGFKRTGSALHRFSTSRMSHGGFASQSTAALTRLMATTDTMRDLGDQNFDFLFQATLLYAQITTTVARDGWITSCTDHYHIACKSCLRPIEEITLDSSMDYTPPDVSHVLKTWRNGEGSWGQEIKQIYPLEGNWKNLAPAEQSYQVGRCIGFLYGDLAYRKSTHAEDSSLFPLSIQGRIRGRGFLKGLLDGLMRASCCQVIHRRSLAHLKRPANAVYGGLIYLIDKLSVSPPFLSLTRSGPIRDELETIPHKIPTSYPTSNRDMGVIVRNYFKYQCRLIEKGKYRSHYSQLWLFSDVLSIDFIGPFSISTTLLQILYKPFLSGKDKNELRELANLSSLLRSGEGWEDIHVKFFTKDILLCPEEIRHACKFGIAKDNNKDMSYPPWGRESRGTITTIPVYYTTTPYPKMLEMPPRIQNPLLSGIRLGQLPTGAHYKIRSILHGMGIHYRDFLSCGDGSGGMTAALLRENVHSRGIFNSLLELSGSVMRGASPEPPSALETLGGDKSRCVNGETCWEYPSDLCDPRTWDYFLRLKAGLGLQIDLIVMDMEVRDSSTSLKIETNVRNYVHRILDEQGVLIYKTYGTYICESEKNAVTILGPMFKTVDLVQTEFSSSQTSEVYMVCKGLKKLIDEPNPDWSSINESWKNLYAFQSSEQEFARAKKVSTYFTLTGIPSQFIPDPFVNIETMLQIFGVPTGVSHAAALKSSDRPADLLTISLFYMAIISYYNINHIRVGPIPPNPPSDGIAQNVGIAITGISFWLSLMEKDIPLYQQCLAVIQQSFPIRWEAVSVKGGYKQKWSTRGDGLPKDTRISDSLAPIGNWIRSLELVRNQVRLNPFNEILFNQLCRTVDNHLKWSNLRRNTGMIEWINRRISKEDRSILMLKSDLHEENSWRD

SEQ ID NO: 19 - protein, 2109 aa, synthetic construct
MEVHDFETDEFNDFNEDDYATREFLNPDERMTYLNHADYNLNSPLISDDIDNLIRKFNSLPIPSMWDSKNWDGVLEMLTSCQANPIPTSQMHKWMGSWLMSDNHDASQGYSFLHEVDKEAEITFDVVETFIRGWGNKPIEYIKKERWTDSFKILAYLCQKFLDLHKLTLILNAVSEVELLNLARTFKGKVRRSSHGTNICRIRVPSLGPTFISEGWAYFKKLDILMDRNFLLMVKDVIIGRMQTVLSMVCRIDNLFSEQDIFSLLNIYRIGDKIVERQGNFSYDLIKMVEPICNLKLMKLARESRPLVPQFPHFENHIKTSVDEGAKIDRGIRFLHDQIMSVKTVDLTLVIYGSFRHWGHPFIDYYTGLEKLHSQVTMKKDIDVSYAKALASDLARIVLFQQFNDHKKWFVNGDLLPHDHPFKSHVKENTWPTAAQVQDFGDKWHELPLIKCFEIPDLLDPSIIYSDKSHSMNRSEVLKHVRMNPNTPIPSKKVLQTMLDTKATNWKEFLKEIDEKGLDDDDLIIGLKGKERELKLAGRFFSLMSWKLREYFVITEYLIKTHFVPMFKGLTMADDLTAVIKKMLDSSSGQGLKSYEAICIANHIDYEKWNNHQRKLSNGPVFRVMGQFLGYPSLIERTHEFFEKSLIYYNGRPDLMRVHNNTLINSTSQRVCWQGQEGGLEGLRQKGWSILNLLVIQREAKIRNTAVKVLAQGDNQVICTQYKTKKSRNVVELQGALNQMVSNNEKIMTAIKIGTGKLGLLINDDETMQSADYLNYGKIPIFRGVIRGLETKRWSRVTCVTNDQIPTCANIMSSVSTNALTVAHFAENPINAMIQYNYFGTFARLLLMMHDPALRQSLYEVQDKIPGLHSSTFKYAMLYLDPSIGGVSGMSLSRFLIRAFPDPVTESLSFWRFIHVHARSEHLKEMSAVFGNPEIAKFRITHIDKLVEDPTSLNIAMGMSPANLLKTEVKKCLIESRQTIRNQVIKDATIYLYHEEDRLRSFLWSINPLFPRFLSEFKSGTFLGVADGLISLFQNSRTIRNSFKKKYHRELDDLIVRSEVSSLTHLGKLHLRRGSCKMWTCSATHADTLRYKSWGRTVIGTTVPHPLEMLGPQHRKETPCAPCNTSGFNYVSVHCPDGIHDVFSSRGPLPAYLGSKTSESTSILQPWERESKVPLIKRATRLRDAISWFVEPDSKLAMTILSNIHSLTGEEWTKRQHGFKRTGSALHRFSTSRMSHGGFASQSTAALTRLMATTDTMRDLGDQNFDFLFQATLLYAQITTTVARDGWITSCTDHYHIACKSCLRPIEEITLDSSMDYTPPDVSHVLKTWRNGEGSWGQEIKQIYPLEGNWKNLAPAEQSYQVGRCIGFLYGDLAYRKSTHAEDSSLFPLSIQGRIRGRGFLKGLLDGLMRASCCQVIHRRSLAHLKRPANAVYGGLIYLIDKLSVSPPFLSLTRSGPIRDELETIPHKIPTSYPTSNRDMGVIVRNYFKYQCRLIEKGKYRSHYSQLWLFSDVLSIDFIGPFSISTTLLQILYKPFLSGKDKNELRELANLSSLLRSGEGWEDIHVKFFTKDILLCPEEIRHACKFGIAKDNNKDMSYPPWGRESRGTITTIPVYYTTTPYPKMLEMPPRIQNPLLSGIRLGQLPTGAHYKIRSILHGMGIHYRDFLSCGDGSGGMTAALLRENVHSRGIFNSLLELSGSVMRGASPEPPSALETLGGDKSRCVNGETCWEYPSDLCDPRTWDYFLRLKAGLGLQIDLIVMDMEVRDSSTSLKIETNVRNYVHRILDEQGVLIYKTYGTYICESEKNAVTILGPMFKTVDLVQTEFSSSQTSEVYMVCKGLKKLIDEPNPDWSSINESWKNLYAFQSSEQEFARAKKVSTYFTLTGIPSQFIPDPFVNIETMLQIFGVPTGVSHAAALKSSDRPADLLTISLFYMAIISYYNINHIRVGPIPPNPPSDGIAQNVGIAITGISFWLSLMEKDIPLYQQCLAVIQQSFPIRWEAVSVKGGYKQKWSTRGDGLPKDTRISDSLAPIGNWIRSLELVRNQVRLNPFNEILFNQLCRTVDNHLKWSNLRRNTGMIEWINRRISKEDRSILMLKSDLHEENSWRD

SEQ ID NO: 20 - protein, 675 aa, synthetic construct
MELAALCRWGLLLALLPPGAASTQVCTGTDMKLRLPASPETHLDMLRHLYQGCQVVQGNLELTYLPTNASLSFLQDIQEVQGYVLIAHNQVRQVPLQRLRIVRGTQLFEDNYALAVLDNGDPLNNTTPVTGASPGGLRELQLRSLTEILKGGVLIQRNPQLCYQDTILWKDIFHKNNQLALTLIDTNRSRACHPCSPMCKGSRCWGESSEDCQSLTRTVCAGGCARCKGPLPTDCCHEQCAAGCTGPKHSDCLACLHFNHSGICELHCPALVTYNTDTFESMPNPEGRYTFGASCVTACPYNYLSTDVGSCTLVCPLHNQEVTAEDGTQRCEKCSKPCARVCYGLGMEHLREVRAVTSANIQEFAGCKKIFGSLAFLPESFDGDPASNTAPLQPEQLQVFETLEEITGYLYISAWPDSLPDLSVFQNLQVIRGRILHNGAYSLTLQGLGISWLGLRSLRELGSGLALIHHNTHLCFVHTVPWDQLFRNPHQALLHTANRPEDECVGEGLACHQLCARGHCWGPGPTQCVNCSQFLRGQECVEECRVLQGLPREYVNARHCLPCHPECQPQNGSVTCFGPEADQCVACAHYKDPPFCVARCPSGVKPDLSYMPIWKFPDEEGACQPCPINCTHSCVDLDDKGCPAEQRASPLTSIISAVVGILLVVVLGVVFGILI

SEQ ID NO: 21 - protein, 668 aa, synthetic construct
MRPSGTAGAALLALLAALCPASRALEEKKVCQGTSNKLTQLGTFEDHFLSLQRMFNNCEVVLGNLEITYVQRNYDLSFLKTIQEVAGYVLIALNTVERIPLENLQIIRGNMYYENSYALAVLSNYDANKTGLKELPMRNLQEILHGAVRFSNNPALCNVESIQWRDIVSSDFLSNMSMDFQNHLGSCQKCDPSCPNGSCWGAGEENCQKLTKIICAQQCSGRCRGKSPSDCCHNQCAAGCTGPRESDCLVCRKFRDEATCKDTCPPLMLYNPTTYQMDVNPEGKYSFGATCVKKCPRNYVVTDHGSCVRACGADSYEMEEDGVRKCKKCEGPCRKVCNGIGIGEFKDSLSINATNIKHFKNCTSISGDLHILPVAFRGDSFTHTPPLDPQELDILKTVKEITGFLLIQAWPENRTDLHAFENLEIIRGRTKQHGQFSLAVVSLNITSLGLRSLKEISDGDVIISGNKNLCYANTINWKKLFGTSGQKTKIISNRGENSCKATGQVCHALCSPEGCWGPEPRDCVSCRNVSRGRECVDKCNLLEGEPREFVENSECIQCHPECLPQAMNITCTGRGPDNCIQCAHYIDGPHCVKTCPAGVMGENNTLVWKYADAGHVCHLCHPNCTYGCTGPGLEGCPTNGPKIPSIATGMVGALLLLLVVALGIGLFM

SEQ ID NO: 22 - protein, 346 aa, synthetic construct
MSSPTSSASSFSSSAPFLASAVSAQPPLPDQCPALCECSEAARTVKCVNRNLTEVPTDLPAYVRNLFLTGNQLAVLPAGAFARRPPLAELAALNLSGSRLDEVRAGAFEHLPSLRQLDLSHNPLADLSPFAFSGSNASVSAPSPLVELILNHIVPPEDERQNRSFEGMVVAALLAGRALQGLRRLELASNHFLYLPRDVLAQLPSLRHLDLSNNSLVSLTYVSFRNLTHLESLHLEDNALKVLHNGTLAELQGLPHIRVFLDNNPWVCDCHMADMVTWLKETEVVQGKDRLTCAYPEKMRNRVLLELNSADLDCDPILPPSLQTSYVFLGIVLALIGAIFLLVLYL

SEQ ID NO: 23 - protein, 487 aa, synthetic construct
MLRRRGSPGMGVHVGAALGALWFCLTGALEVQVPEDPVVALVGTDATLCCSFSPEPGFSLAQLNLIWQLTDTKQLVHSFAEGQDQGSAYANRTALFPDLLAQGNASLRLQRVRVADEGSFTCFVSIRDFGSAAVSLQVAAPYSKPSMTLEPNKDLRPGDTVTITCSSYQGYPEAEVFWQDGQGVPLTGNVTTSQMANEQGLFDVHSILRVVLGANGTYSCLVRNPVLQQDAHSSVTITPQRSPTGAVEVQVPEDPVVALVGTDATLRCSFSPEPGFSLAQLNLIWQLTDTKQLVHSFTEGRDQGSAYANRTALFPDLLAQGNASLRLQRVRVADEGSFTCFVSIRDFGSAAVSLQVAAPYSKPSMTLEPNKDLRPGDTVTITCSSYRGYPEAEVFWQDGQGVPLTGNVTTSQMANEQGLFDVHSVLRVVLGANGTYSCLVRNPVLQQDAHGSVTITGQPMTFPPEALWVTVGLSVCLIALLVALAFV

SEQ ID NO: 24 - protein, 297 aa, synthetic construct
MARGPGLAPPPLRLPLLLLVLAAVTGHTAAQDNCTCPTNKMTVCSPDGPGGRCQCRALGSGMAVDCSTLTSKCLLLKARMSAPKNARTLVRPSEHALVDNDGLYDPDCDPEGRFKARQCNQTSVCWCVNSVGVRRTDKGDLSLRCDELVRTHHILIDLRHRPTAGAFNHSDLDAELRRLFRERYRLHPKFVAAVHYEQPTIQIELRQNTSQKAAGDVDIGDAAYYFERDIKGESLFQGRGGLDLRVRGEPLQVERTLIYYLDEIPPKFSMKRLTAGLIAVIVVVVVALVAGMAVLVI

SEQ ID NO: 25 - protein, 77 aa, synthetic construct
MLQMAGQCSQNEYFDSLLHACIPCQLRCSSNTPPLTCQRYCNASVTNSVKGTNAILWTCLGLSLIISLAVFVLMFLL

SEQ ID NO: 26 - protein, 785 aa, synthetic construct
MQSKVLLAVALWLCVETRAASVGLPSVSLDLPRLSIQKDILTIKANTTLQITCRGQRDLDWLWPNNQSGSEQRVEVTECSDGLFCKTLTIPKVIGNDTGAYKCFYRETDLASVIYVYVQDYRSPFIASVSDQHGVVYITENKNKTVVIPCLGSISNLNVSLCARYPEKRFVPDGNRISWDSKKGFTIPSYMISYAGMVFCEAKINDESYQSIMYIVVVVGYRIYDVVLSPSHGIELSVGEKLVLNCTARTELNVGIDFNWEYPSSKHQHKKLVNRDLKTQSGSEMKKFLSTLTIDGVTRSDQGLYTCAASSGLMTKKNSTFVRVHEKPFVAFGSGMESLVEATVGERVRIPAKYLGYPPPEIKWYKNGIPLESNHTIKAGHVLTIMEVSERDTGNYTVILTNPISKEKQSHVVSLVVYVPPQIGEKSLISPVDSYQYGTTQTLTCTVYAIPPPHHIHWYWQLEEECANEPSQAVSVTNPYPCEEWRSVEDFQGGNKIEVNKNQFALIEGKNKTVSTLVIQAANVSALYKCEAVNKVGRGERVISFHVTRGPEITLQPDMQPTEQESVSLWCTADRSTFENLTWYKLGPQPLPIHVGELPTPVCKNLDTLWKLNATMFSNSTNDILIMELKNASLQDQGDYVCLAQDRKTKKRHCVVRQLTVLERVAPTITGNLENQTTSIGESIEVSCTASGNPPPQIMWFKDNETLVEDSGIVLKDGNRNLTIRRVRKEDEGLYTCQACSVLGCAKVEAFFIIEGAQEKTNLEIIILVGTAVIAMFFWLLLVII

SEQ ID NO: 27 - protein, 247 aa, synthetic construct
MAGSPTCLTLIYILWQLTGSAASGPVKELVGSVGGAVTFPLKSKVKQVDSIVWTFNTTPLVTIQPEGGTIIVTQNRNRERVDFPDGGYSLKLSKLKKNDSGIYYVGIYSSSLQQPSTQEYVLHVYEHLSKPKVTMGLQSNKNGTCVTNLTCCMEHGEEDVIYTWKALGQAANESHNGSILPISWRWGESDMTFICVARNPVSRNFSSPILARKLCEGAADDPDSSMVLLCLLLVPLLLSLFVLGLFL

SEQ ID NO: 28 - protein, 323 aa, synthetic construct
MPPPRLLFFLLFLTPMEVRPEEPLVVKVEEGDNAVLQCLKGTSDGPTQQLTWSRESPLKPFLKLSLGLPGLGIHMRPLAIWLFIFNVSQQMGGFYLCQPGPPSEKAWQPGWTVNVEGSGELFRWNVSDLGGLGCGLKNRSSEGPSSPSGKLMSPKLYVWAKDRPEIWEGEPPCLPPRDSLNQSLSQDLTMAPGSTLWLSCGVPPDSVSRGPLSWTHVHPKGPKSLLSLELKDDRPARDMWVMETGLLLPRATAQDAGKYYCHRGNLTMSFHLEITARPVLWHWLLRTGGWKVSAVTLAYLIFCLCSLVGILHLQRALVLRRKR

SEQ ID NO: 29 - protein, 295 aa, synthetic construct
MPEEPLVVKVEEGDNAVLQCLKGTSDGPTQQLTWSRESPLKPFLKLSLGLPGLGIHMRPLAIWLFIFNVSQQMGGFYLCQPGPPSEKAWQPGWTVNVEGSGELFRWNVSDLGGLGCGLKNRSSEGPSSPSGKLMSPKLYVWAKDRPEIWEGEPPCLPPRDSLNQSLSQDLTMAPGSTLWLSCGVPPDSVSRGPLSWTHVHPKGPKSLLSLELKDDRPARDMWVMETGLLLPRATAQDAGKYYCHRGNLTMSFHLEITARPVLWHWLLRTGGWKVSAVTLAYLIFCLCSLVGILHL

SEQ ID NO: 30 - protein, 229 aa, synthetic construct
MARLALSPVPSHWMVALLLLLSAEPVPAARSEDRYRNPKGSACSRIWQSPRFIARKRGFTVKMHCYMNSASGNVSWLWKQEMDENPQQLKLEKGRMEESQNESLATLTIQGIRFEDNGIYFCQQKCNNTSEVYQGCGTELRVMGFSTLAQLKQRNTLKDGIIMIQTLLIILFIIVPIFLLLDKDDSKAGMEEDHTYEGLDIDQTATYEDIVTLRTGEVKWSVGEHPGQE

SEQ ID NO: 31 - protein, 580 aa, synthetic construct
MAGTVRTACLVVAMLLSLDFPGQAQPPPPPPDATCHQVRSFFQRLQPGLKWVPETPVPGSDLQVCLPKGPTCCSRKMEEKYQLTARLNMEQLLQSASMELKFLIIQNAAVFQEAFEIVVRHAKNYTNAMFKNNYPSLTPQAFEFVGEFFTDVSLYILGSDINVDDMVNELFDSLFPVIYTQLMNPGLPDSALDINECLRGARRDLKVFGNFPKLIMTQVSKSLQVTRIFLQALNLGIEVINTTDHLKFSKDCGRMLTRMWYCSYCQGLMMVKPCGGYCNVVMQGCMAGVVEIDKYWREYILSLEELVNGMYRIYDMENVLLGLFSTIHDSIQYVQKNAGKLTTTIGKLCAHSQQRQYRSAYYPEDLFIDKKVLKVAHVEHEETLSSRRRELIQKLKSFISFYSALPGYICSHSPVAENDTLCWNGQELVERYSQKAARNGMKNQFNLHELKMKGPEPVVSQIIDKLKHINQLLRTMSMPKGRVLDKNLDEEGFESGDCGDDEDECIGGSGDGMIKVKNQLRFLAELAYDLDVDDAPGNSQQATPKDNEISTFHNLGNVHSPLKLLTSMAISVVCFFFLVH

SEQ ID NO: 32 - protein, 580 aa, synthetic construct
MAGTVRTACLVVAMLLSLDFPGQAQPPPPPPDATCHQVRSFFQRLQPGLKWVPETPVPGSDLQVCLPKGPTCCSRKMEEKYQLTARLNMEQLLQSASMELKFLIIQNAAVFQEAFEIVVRHAKNYTNAMFKNNYPSLTPQAFEFVGEFFTDVSLYILGSDINVDDMVNELFDSLFPVIYTQLMNPGLPDSALDINECLRGARRDLKVFGNFPKLIMTQVSKSLQVTRIFLQALNLGIEVINTTDHLKFSKDCGRMLTRMWYCSYCQGLMMVKPCGGYCNVVMQGCMAGVVEIDKYWREYILSLEELVNGMYRIYDMENVLLGLFSTIHDSIQYVQKNAGKLTTTIGKLCAHSQQRQYSSAYYPEDLFIDKKVLKVAHVEHEETLSSRRRELIQKLKSFISFYSALPGYICSHSPVAENDTLCWNGQELVERYSQKAARNGMKNQFNLHELKMKGPEPVVSQIIDKLKHINQLLRTMSMPKGRVLDKNLDEEGFESGDCGDDEDECIGGSGDGMIKVKNQLRFLAELAYDLDVDDAPGNSQQATPKDNEISTFHNLGNVHSPLKLLTSMAISVVCFFFLVH

SEQ ID NO: 33 - protein, 578 aa, synthetic construct
MAGTVRTACLVVAMLLSLDFPGQAQPPPPPPDATCHQVRSFFQRLQPGLKWVPETPVPGSDLQVCLPKGPTCCSRKMEEKYQLTARLNMEQLLQSASMELKFLIIQNAAVFQEAFEIVVRHAKNYTNAMFKNNYPSLTPQAFEFVGEFFTDVSLYILGSDINVDDMVNELFDSLFPVIYTQLMNPGLPDSALDINECLRGARRDLKVFGNFPKLIMTQVSKSLQVTRIFLQALNLGIEVINTTDHLKFSKDCGRMLTRMWYCSYCQGLMMVKPCGGYCNVVMQGCMAGVVEIDKYWREYILSLEELVNGMYRIYDMENVLLGLFSTIHDSIQYVQKNAGKLTTTIGKLCAHSQQRQSAYYPEDLFIDKKVLKVAHVEHEETLSSRRRELIQKLKSFISFYSALPGYICSHSPVAENDTLCWNGQELVERYSQKAARNGMKNQFNLHELKMKGPEPVVSQIIDKLKHINQLLRTMSMPKGRVLDKNLDEEGFESGDCGDDEDECIGGSGDGMIKVKNQLRFLAELAYDLDVDDAPGNSQQATPKDNEISTFHNLGNVHSPLKLLTSMAISVVCFFFLVH

SEQ ID NO: 34 - protein, 169 aa, synthetic construct
MDQWSTQDLYNNPVTAVFNYQGLWRSCVRESSGFTECRGYFTLLGLPAMLQAVRALMIVGIVLGAIGLLVSIFALKCIRIGSMEDSAKANMTLTSGIMFIVSGLCAIAGVSVFANMLVTNFWMSTANMYTGMGGMVQTVQTRYTFGAALFVGWVAGGLTLIGGVMMCIA

SEQ ID NO: 35 - protein, 121 aa, synthetic construct
MDQWSTQDLYNNPVTAVFNYQGLWRSCVRESSGFTECRGYFTLLGLPAMLQAVRGGGGSGGGGSGGGGSVTNFWMSTANMYTGMGGMVQTVQTRYTFGAALFVGWVAGGLTLIGGVMMCIA

SEQ ID NO: 36 - protein, 395 aa, synthetic construct
MTDRQTDTAPSPSYHLLPGRRRTVDAAASRGQGPEPAPGGGVEGVGARGVALKLFVQLLGCSRFGGAVVRAGEAEPSGAARSASSGREEPQPEEGEEEEEKEEERGPQWRLGARKPGSWTGEAAVCADSAPAARAPQALARASGRGGRVARRGAEESGPPHSPSRRGSASRAGPGRASETMNFLLSWVHWSLALLLYLHHAKWSQAAPMAEGGGQNHHEVVKFMDVYQRSYCHPIETLVDIFQEYPDEIEYIFKPSCVPLMRCGGCCNDEGLECVPTEESNITMQIMRIKPHQGQHIGEMSFLQHNKCECRPKKDRARQEKKSVRGKGKGQKRKRKKSRYKSWSVPCGPCSERRKHLFVQDPQTCKCSCKNTDSRCKARQLELNERTCRCDKPRR

SEQ ID NO: 37 - protein, 664 aa, synthetic construct
MRANDALQVLGLLFSLARGSEVGNSQAVCPGTLNGLSVTGDAENQYQTLYKLYERCEVVMGNLEIVLTGHNADLSFLQWIREVTGYVLVAMNEFSTLPLPNLRVVRGTQVYDGKFAIFVMLNYNTNSSHALRQLRLTQLTEILSGGVYIEKNDKLCHMDTIDWRDIVRDRDAEIVVKDNGRSCPPCHEVCKGRCWGPGSEDCQTLTKTICAPQCNGHCFGPNPNQCCHDECAGGCSGPQDTDCFACRHFNDSGACVPRCPQPLVYNKLTFQLEPNPHTKYQYGGVCVASCPHNFVVDQTSCVRACPPDKMEVDKNGLKMCEPCGGLCPKACEGTGSGSRFQTVDSSNIDGFVNCTKILGNLDFLITGLNGDPWHKIPALDPEKLNVFRTVREITGYLNIQSWPPHMHNFSVFSNLTTIGGRSLYNRGFSLLIMKNLNVTSLGFRSLKEISAGRIYISANRQLCYHHSLNWTKVLRGPTEERLDIKHNRPRRDCVAEGKVCDPLCSSGGCWGPGPGQCLSCRNYSRGGVCVTHCNFLNGEPREFAHEAECFSCHPECQPMEGTATCNGSGSDTCAQCAHFRDGPHCVSSCPHGVLGAKGPIYKYPDVQNECRPCHENCTQGCKGPELQDCLGQTLVLIGKTHLTMALTVIAGLVVIFMMLGGTFL

SEQ ID NO: 38 - protein, 180 aa, synthetic construct
MQAEGRGTGGSTGDADGPGGPGIPDGPGGNAGGPGEAGATGGRGPRGAGAARASGPGGGAPRGPHGGAASGLNGCCRCGARGPESRLLEFYLAMPFATPMEAELARRSLAQDAPPLPVPGVLLKEFTVSGNILTIRLTAADHRQLQLSISSCLQQLSLLMWITQCFLPVFLAQPPSGQRR

SEQ ID NO: 39 - protein, 336 aa, synthetic construct
MEVEKTACPSGKKAREIDESLIFYKKWELEACVDAALLATQMDRVNAIPFTYEQLDVLKHKLDELYPQGYPESVIQHLGYLFLKMSPEDIRKWNVTSLETLKALLEVDKGHEMSPQAPRRPLPQVATLIDRFVKGRGQLDKDTLDTLTAFYPGYLCSLSPEELSSVPPSSIWAVRPQDLDTCDPRQLDVLYPKARLAFQNMNGSEYFVKIQSFLGGAPTEDLKALSQQNVSMDLATFMKLRTDAVLPLTVAEVQKLLGPHVEGLKAEERHRPVRDWILRQRQDDLDTLGLGLQGGIPNGYLVLDLSVQETLSGTPCLLGPGPVLTVLALLLASTLA

SEQ ID NO: 40 - protein, 407 aa, synthetic construct
MRVLLAALGLLFLGALRAFPQDRPFEDTCHGNPSHYYDKAVRRCCYRCPMGLFPTQQCPQRPTDCRKQCEPDYYLDEADRCTACVTCSRDDLVEKTPCAWNSSRVCECRPGMFCSTSAVNSCARCFFHSVCPAGMIVKFPGTAQKNTVCEPASPGVSPACASPENCKEPSSGTIPQAKPTPVSPATSSASTMPVRGGTRLAQEAASKLTRAPDSPSSVGRPSSDPGLSPTQPCPEGSGDCRKQCEPDYYLDEAGRCTACVSCSRDDLVEKTPCAWNSSRTCECRPGMICATSATNSCARCVPYPICAAETVTKPQDMAEKDTTFEAPPLGTQPDCNPTPENGEAPASTSPTQSLLVDSQASKTLPIPTSAPVALSSTGKPVLDAGPVLFWVILVLVVVVGSSAFLLC

SEQ ID NO: 41 - protein, 1125 aa, synthetic construct
MSGHASSTPGGEKETSATQRSSVPSSTEKNAVSMTSSVLSSHSPGSGSSTTQGQDVTLAPATEPASGSAATWGQDVTSVPVTRPALGSTTPPAHDVTSAPDNKPAPGSTAPPAHGVTSAPDTRPAPGSTAPQAHGVTSAPDTRPAPGSTAPPAHGVTSAPDTRPAPGSTAPPAHGVTSAPDTRPAPGSTAPAAHGVTSAPDTRPAPGSTAPQAHGVTSAPDTRPAPGSTAPPAHGVTSAPDTRPAPGSTAPPAHGVTSAPDTRPAPGSTAPPAHGVTSAPESRPAPGSTAPAAHGVTSAPESRPAPGSTAPAAHGVTSAPESRPAPGSTAPPAHGVTSAPDTRPAPGSTAPPAHGVTSAPDTRPAPGSTAPPAHGVTSAPDTRPAPGSTAPPAHGVTSAPDTRPAPGSTAPPAHGVTSAPESRPAPGSTAPPAHGVTSAPESRPAPGSTAPAAHGVTSAPESRPAPGSTAPAAHGVTSAPESRPAPGSTAPRAHGVTSAPDTRPAPGSTAPPAHGVTSAPDTRPAPGSTAPPAHGVTSAPDTRPAPGSTAPPAHGVTSAPDTRPAPGSTAPPAHGVTSAPDTRPAPGSTAPPAHGVTSAPDTRPAPGSTAPPAHGVTSAPDTRPAPGSTAPAAHGVTSAPESRPAPGSTAPAAHGVTSAPESRPAPGSTAPPAHGVTSAPDTRPAPGSTAPPAHGVTSAPDTRPAPGSTAPPAHGVTSAPDTRPAPGSTAPPAHGVTSAPDTRPAPGSTAPPAHGVTSAPDTRPAPGSTAPPAHGVTSAPDTRPAPGSTAPPAHGVTSAPDTRPAPGSTAPPAHGVTSAPDTRPAPGSTAPPAHGVTSAPDTRRAPGSTPAPGSTAPPAHGVTSAPDTRPAPGSTAPPAHGVTSAPDNRPALGSTAPPVHNVTSASGSASGSASTLVHNGTSARATTTPASKSTPFSIPSHHSDTPTTLASHSTKTDASSTHHSTVPPLTSSNHSTSPQLSTGVSFFFLSFHISNLQFNSSLEDPSTDYYQELQRDISEMFLQIYKQGGFLGLSNIKFRPGSVVVQLTLAFREGTINVHDVETQFNQYKTEAASRYNLTISDVSVSDVPFPFSAQSGAGVPGWGIALLVLVCVLVALAIVYLIAL

SEQ ID NO: 42 - protein, 317 aa, synthetic construct
MSSEQKSQHCKPEEGVEAQEEALGLVGAQAPTTEEQEAAVSSSSPLVPGTLEEVPAAESAGPPQSPQGASALPTTISFTCWRQPNEGSSSQEEEGPSTSPDAESLFREALSNKVDELAHFLLRKYRAKELVTKAEMLERVIKNYKRCFPVIFGKASESLKMIFGIDVKEVDPASNTYTLVTCLGLSYDGLLGNNQIFPKTGLLIIVLGTIAMEGDSASEEEIWEELGVMGVYDGREHTVYGEPRKLLTQDWVQENYLEYRQVPGSNPARYEFLWGPRALAETSYVKVLEHVVRVNARVRIAYPSLREAALLEEEEGV

SEQ ID NO: 43 - protein, 317 aa, synthetic construct
MSSEQKSQHCKPEEGVEAQEEALGLVGAQAPTTEEQEAAVSSSSPLVPGTLEEVPAAESAGPPQSPQGASALPTTISFTCWRQPNEGSSSQEEEGPSTSPDAESLFREALSNKVDELAHFLLRKYRAKELVTKAEMLERVIKNYKRCFPVIFGKASESLKMIFGIDVKEVDPTSNTYTLVTCLGLSYDGLLGNNQIFPKTGLLIIVLGTIAMEGDSASEEEIWEELGVMGVYDGREHTVYGEPRKLLTQDWVQENYLEYRQVPGSNPARYEFLWGPRALAETSYVKVLEHVVRVNARVRIAYPSLREAALLEEEEGV

SEQ ID NO: 44 - protein, 931 aa, synthetic construct
ECKEALAKSEMNVNMKYQLPNFTAETPIQNVILHEHHIFLGATNYIYVLNEEDLQKVAEYKTGPVLEHPDCFPCQDCSSKANLSGGVWKDNINMALVVDTYYDDQLISCGSVNRGTCQRHVFPHNHTADIQSEVHCIFSPQIEEPSQCPDCVVSALGAKVLSSVKDRFINFFVGNTINSSYFPDHPLHSISVRRLKETKDGFMFLTDQSYIDVLPEFRDSYPIKYVHAFESNNFIYFLTVQRETLDAQTFHTRIIRFCSINSGLHSYMEMPLECILTEKRKKRSTKKEVFNILQAAYVSKPGAQLARQIGASLNDDILFGVFAQSKPDSAEPMDRSAMCAFPIKYVNDFFNKIVNKNNVRCLQHFYGPNHEHCFNRTLLRNSSGCEARRDEYRTEFTTALQRVDLFMGQFSEVLLTSISTFIKGDLTIANLGTSEGRFMQVVVSRSGPSTPHVNFLLDSHPVSPEVIVEHTLNQNGYTLVITGKKITKIPLNGLGCRHFQSCSQCLSAPPFVQCGWCHDKCVRSEECLSGTWTQQICLPAIYKVFPNSAPLEGGTRLTICGWDFGFRRNNKFDLKKTRVLLGNESCTLTLSESTMNTLKCTVGPAMNKHFNMSIIISNGHGTTQYSTFSYVDPVITSISPKYGPMAGGTLLTLTGNYLNSGNSRHISIGGKTCTLKSVSNSILECYTPAQTISTEFAVKLKIDLANRETSIFSYREDPIVYEIHPTKSFISGGSTITGVGKNLNSVSVPRMVINVHEAGRNFTVACQHRSNSEIICCTTPSLQQLNLQLPLKTKAFFMLDGILSKYFDLIYVHNPVFKPFEKPVMISMGNENVLEIKGNDIDPEAVKGEVLKVGNKSCENIHLHSEAVLCTVPNDLLKLNSELNIEWKQAISSTVLGKVIVQPDQNFTGLIAGVVSISTALLLLLGFFLWL

SEQ ID NO: 45 - protein, 706 aa, synthetic construct
MHLLGPWLLLLVLEYLAFSDSSKWVFEHPETLYAWEGACVWIPCTYRALDGDLESFILFHNPEYNKNTSKFDGTRLYESTKDGKVPSEQKRVQFLGDKNKNCTLSIHPVHLNDSGQLGLRMESKTEKWMERIHLNVSERPFPPHIQLPPEIQESQEVTLTCLLNFSCYGYPIQLQWLLEGVPMRQAAVTSTSLTIKSVFTRSELKFSPQWSHHGKIVTCQLQDADGKFLSNDTVQLNVKHTPKLEIKVTPSDAIVREGDSVTMTCEVSSSNPEYTTVSWLKDGTSLKKQNTFTLNLREVTKDQSGKYCCQVSNDVGPGRSEEVFLQVQYAPEPSTVQILHSPAVEGSQVEFLCMSLANPLPTNYTWYHNGKEMQGRTEEKVHIPKILPWHAGTYSCVAENILGTGQRGPGAELDVQYPPKKVTTVIQNPMPIREGDTVTLSCNYNSSNPSVTRYEWKPHGAWEEPSLGVLKIQNVGWDNTTIACAACNSWCSWASPVALNVQYAPRDVRVRKIKPLSEIHSGNSVSLQCDFSSSHPKEVQFFWEKNGRLLGKESQLNFDSISPEDAGSYSCWVNNSIGQTASKAWTLEVLYAPRRLRVSMSPGDQVMEGKSATLTCESDANPPVSHYTWFDWNNQSLPYHSQKLRLEPVKVQHSGAYWCQGTNSVGKGRSPLSTLTVYYSPETIGRRVAVGLGSCLAILILAICGL

SEQ ID NO: 46 - protein, 134 aa, synthetic construct
MAPTSSSTKKTQLQLEHLLLDLQMILNGINNYKNPKLTRMLTCKFYMPKKATELKHLQCLEEELKPLEECLNLAQSKNFHLRPRDLISNINVIVLELKGSETTFMCEYADETATIVEFLNRWITFAQSIISTLT

SEQ ID NO: 47 - protein, 319 aa, synthetic construct
MAPTSSSTKKTQLQLEHLLLDLQMILNGINNYKNCKLTRMLTFKFYMPKKATELKHLQCLEEELKPLEEVLNLAQSKNFHLRPRDLISNINVIVLELKGSETTFMCEYADETATIVEFLNRWITFAQSIISTLTATNFSLLKQAGDVEENPGPMELCCDDPPEIPHATFKAMAYKEGTMLNCECKRGFRRIKSGSLYMLCTGNSSHSSWDNQCQCTSSATRNTTKQVTPQPEEQKERKTTEMQSPMQPVDQASLPGHCREPPPWENEATERIYHFVVGQMVYYQCVQGYRALHRGPAESVCKMTHGKTRWTQPQLICTG

SEQ ID NO: 48 - protein, 253 aa, synthetic construct
MWPPGSASQPPPSPAAATGLHPAARPVSLQCRLSMCPARSLLLVATLVLLDHLSLARNLPVATPDPGMFPCLHHSQNLLRAVSNMLQKARQTLEFYPCTSEEIDHEDITKDKTSTVEACLPLELTKNESCLNSRETSFITNGSCLASRKTSFMMALCLSSIYEDLKMYQVEFKTMNAKLLMDPKRQIFLDQNMLAVIDELMQALNFNSETVPQKSSLEEPDFYKTKIKLCILLHAFRIRAVTIDRVMSYLNAS

SEQ ID NO: 49 - protein, 328 aa, synthetic construct
MCHQQLVISWFSLVFLASPLVAIWELKKDVYVVELDWYPDAPGEMVVLTCDTPEEDGITWTLDQSSEVLGSGKTLTIQVKEFGDAGQYTCHKGGEVLSHSLLLLHKKEDGIWSTDILKDQKEPKNKTFLRCEAKNYSGRFTCWWLTTISTDLTFSVKSSRGSSDPQGVTCGAATLSAERVRGDNKEYEYSVECQEDSACPAAEESLPIEVMVDAVHKLKYENYTSSFFIRDIIKPDPPKNLQLKPLKNSRQVEVSWEYPDTWSTPHSYFSLTFCVQVQGKSKREKKDRVFTDKTSATVICRKNASISVRAQDRYYSSSWSEWASVPCS

SEQ ID NO: 50 - protein, 144 aa, synthetic construct
MWLQSLLLLGTVACSISAPARSPSPSTQPWEHVNAIQEARRLLNLSRDTAAEMNETVEVISEMFDLQEPTCLQTRLELYKQGLRGSLTKLKGPLTMMASHYKQHCPPTPETSCATQIITFESFKENLKDFLLVIPFDCWEPVQE

SEQ ID NO: 51 - protein, 153 aa, synthetic construct
MYRMQLLSCIALSLALVTNSAPTSSSTKKTQLQLEHLLLDLQMILNGINNYKNPKLTRMLTFKFYMPKKATELKHLQCLEEELKPLEEVLNLAQSKNFHLRPRDLISNINVIVLELKGSETTFMCEYADETATIVEFLNRWITFCQSIISTLT

SEQ ID NO: 52 - protein, 162 aa, synthetic construct
MRISKPHLRSISIQCYLCLLLNSHFLTEAGIHVFILGCFSAGLPKTEANWVNVISDLKKIEDLIQSMHIDATLYTESDVHPSCKVTAMKCFLLELQVISLESGDASIHDTVENLIILANNSLSSNGNVTESGCKECEELEEKNIKEFLQSFVHIVQMFINTS

SEQ ID NO: 53 - protein, 135 aa, synthetic construct
MVLGTIDLCSCFSAGLPKTEANWVNVISDLKKIEDLIQSMHIDATLYTESDVHPSCKVTAMKCFLLELQVISLESGDASIHDTVENLIILANNSLSSNGNVTESGCKECEELEEKNIKEFLQSFVHIVQMFINTS

SEQ ID NO: 54 - protein, 193 aa, synthetic construct
MAAEPVEDNCINFVAMKFIDNTLYFIAEDDENLESDYFGKLESKLSVIRNLNDQVLFIDQGNRPLFEDMTDSDCRDNAPRTIFIISMYKDSQPRGMAVTISVKCEKISTLSCENKIISFKEMNPPDNIKDTKSDIIFFQRSVPGHDNKMQFESSSYEGYFLACEKERDLFKLILKKEDELGDRSIMFTVQNED

SEQ ID NO: 55 - protein, 189 aa, synthetic construct
MAAEPVEDNCINFVAMKFIDNTLYFIENLESDYFGKLESKLSVIRNLNDQVLFIDQGNRPLFEDMTDSDCRDNAPRTIFIISMYKDSQPRGMAVTISVKCEKISTLSCENKIISFKEMNPPDNIKDTKSDIIFFQRSVPGHDNKMQFESSSYEGYFLACEKERDLFKLILKKEDELGDRSIMFTVQNED

SEQ ID NO: 56 - protein, 233 aa, synthetic construct
MSTESMIRDVELAEEALPKKTGGPQGSRRCLFLSLFSFLIVAGATTLFCLLHFGVIGPQREEFPRDLSLISPLAQAVRSSSRTPSDKPVAHVVANPQAEGQLQWLNRRANALLANGVELRDNQLVVPSEGLYLIYSQVLFKGQGCPSTHVLLTHTISRIAVSYQTKVNLLSAIKSPCQRETPEGAEAKPWYEPIYLGGVFQLEKGDRLSAEINRPDYLDFAESGQVYFGIIAL

SEQ ID NO: 57 - protein, 187 aa, synthetic construct
MTNKCLLQIALLLCFSTTALSMSYNLLGFLQRSSNFQCQKLLWQLNGRLEYCLKDRMNFDIPEEIKQLQQFQKEDAALTIYEMLQNIFAIFRQDSSSTGWNETIVENLLANVYHQINHLKTVLEEKLEKEDFTRGKLMSSLHLKRYYGRILHYLKAKEYSHCAWTIVRVEILRNFYFINRLTGYLRN

SEQ ID NO: 58 - protein, 219 aa, synthetic construct
MCPARSLLLVATLVLLDHLSLARNLPVATPDPGMFPCLHHSQNLLRAVSNMLQKARQTLEFYPCTSEEIDHEDITKDKTSTVEACLPLELTKNESCLNSRETSFITNGSCLASRKTSFMMALCLSSIYEDLKMYQVEFKTMNAKLLMDPKRQIFLDQNMLAVIDELMQALNFNSETVPQKSSLEEPDFYKTKIKLCILLHAFRIRAVTIDRVMSYLNAS

SEQ ID NO: 59 - protein, 239 aa, synthetic construct
MWPPGSASQPPPSPAAATGLHPAARPVSLQCRLSMCPARSLLLVATLVLLDHLSLARNLPVATPDPGMFPCLHHSQNLLRAVSNMLQKARQTLEFYPCTSEEIDHEDITKDKTSTVEACLPLELTKNGSCLASRKTSFMMALCLSSIYEDLKMYQVEFKTMNAKLLMDPKRQIFLDQNMLAVIDELMQALNFNSETVPQKSSLEEPDFYKTKIKLCILLHAFRIRAVTIDRVMSYLNAS

SEQ ID NO: 60 - protein, 215 aa, synthetic construct
MWPPGSASQPPPSPAAATGLHPAARPVSLQCRLSMCPARSLLLVATLVLLDHLSLARNLPVATPDPGMFPCLHHSQNLLRAVSNMLQKNESCLNSRETSFITNGSCLASRKTSFMMALCLSSIYEDLKMYQVEFKTMNAKLLMDPKRQIFLDQNMLAVIDELMQALNFNSETVPQKSSLEEPDFYKTKIKLCILLHAFRIRAVTIDRVMSYLNAS